European Patent Specification EP 3 677 589 B1, published November 26, 2025. Title: IMPROVED MANUFACTURING METHOD OF ANTIBODY-DRUG CONJUGATE. Applicant: DAIICHI SANKYO COMPANY, LIMITED. The sequence listing filed with the application follows.

SEQUENCE LISTING (10 sequences)

SEQ ID NO: 1 - protein, 450 aa, Artificial Sequence
  Heavy chain of anti-HER2 antibody
EVQLVESGGGLVQPGGSLRLSCAASGFNIKDTYIHWVRQAPGKGLEWVARIYPTNGYTRYADSVKGRFTISADTSKNTAYLQMNSLRAEDTAVYYCSRWGGDGFYAMDYWGQGTLVTVSSASTKGPSVFPLAPSSKSTSGGTAALGCLVKDYFPEPVTVSWNSGALTSGVHTFPAVLQSSGLYSLSSVVTVPSSSLGTQTYICNVNHKPSNTKVDKKVEPKSCDKTHTCPPCPAPELLGGPSVFLFPPKPKDTLMISRTPEVTCVVVDVSHEDPEVKFNWYVDGVEVHNAKTKPREEQYNSTYRVVSVLTVLHQDWLNGKEYKCKVSNKALPAPIEKTISKAKGQPREPQVYTLPPSREEMTKNQVSLTCLVKGFYPSDIAVEWESNGQPENNYKTTPPVLDSDGSFFLYSKLTVDKSRWQQGNVFSCSVMHEALHNHYTQKSLSLSPGK

SEQ ID NO: 2 - protein, 214 aa, Artificial Sequence
  Light chain of anti-HER2 antibody
DIQMTQSPSSLSASVGDRVTITCRASQDVNTAVAWYQQKPGKAPKLLIYSASFLYSGVPSRFSGSRSGTDFTLTISSLQPEDFATYYCQQHYTTPPTFGQGTKVEIKRTVAAPSVFIFPPSDEQLKSGTASVVCLLNNFYPREAKVQWKVDNALQSGNSQESVTEQDSKDSTYSLSSTLTLSKADYEKHKVYACEVTHQGLSSPVTKSFNRGEC

SEQ ID NO: 3 - protein, 447 aa, Artificial Sequence
  Heavy chain of anti-HER3 antibody
QVQLQQWGAGLLKPSETLSLTCAVYGGSFSGYYWSWIRQPPGKGLEWIGEINHSGSTNYNPSLKSRVTISVETSKNQFSLKLSSVTAADTAVYYCARDKWTWYFDLWGRGTLVTVSSASTKGPSVFPLAPSSKSTSGGTAALGCLVKDYFPEPVTVSWNSGALTSGVHTFPAVLQSSGLYSLSSVVTVPSSSLGTQTYICNVNHKPSNTKVDKRVEPKSCDKTHTCPPCPAPELLGGPSVFLFPPKPKDTLMISRTPEVTCVVVDVSHEDPEVKFNWYVDGVEVHNAKTKPREEQYNSTYRVVSVLTVLHQDWLNGKEYKCKVSNKALPAPIEKTISKAKGQPREPQVYTLPPSREEMTKNQVSLTCLVKGFYPSDIAVEWESNGQPENNYKTTPPVLDSDGSFFLYSKLTVDKSRWQQGNVFSCSVMHEALHNHYTQKSLSLSPGK

SEQ ID NO: 4 - protein, 220 aa, Artificial Sequence
  Light chain of anti-HER3 antibody
DIEMTQSPDSLAVSLGERATINCRSSQSVLYSSSNRNYLAWYQQNPGQPPKLLIYWASTRESGVPDRFSGSGSGTDFTLTISSLQAEDVAVYYCQQYYSTPRTFGQGTKVEIKRTVAAPSVFIFPPSDEQLKSGTASVVCLLNNFYPREAKVQWKVDNALQSGNSQESVTEQDSKDSTYSLSSTLTLSKADYEKHKVYACEVTHQGLSSPVTKSFNRGEC

SEQ ID NO: 5 - protein, 470 aa, Artificial Sequence
  Heavy chain of anti-TROP2 antibody
MKHLWFFLLLVAAPRWVLSQVQLVQSGAEVKKPGASVKVSCKASGYTFTTAGMQWVRQAPGQGLEWMGWINTHSGVPKYAEDFKGRVTISADTSTSTAYLQLSSLKSEDTAVYYCARSGFGSSYWYFDVWGQGTLVTVSSASTKGPSVFPLAPSSKSTSGGTAALGCLVKDYFPEPVTVSWNSGALTSGVHTFPAVLQSSGLYSLSSVVTVPSSSLGTQTYICNVNHKPSNTKVDKRVEPKSCDKTHTCPPCPAPELLGGPSVFLFPPKPKDTLMISRTPEVTCVVVDVSHEDPEVKFNWYVDGVEVHNAKTKPREEQYNSTYRVVSVLTVLHQDWLNGKEYKCKVSNKALPAPIEKTISKAKGQPREPQVYTLPPSREEMTKNQVSLTCLVKGFYPSDIAVEWESNGQPENNYKTTPPVLDSDGSFFLYSKLTVDKSRWQQGNVFSCSVMHEALHNHYTQKSLSLSPGK

SEQ ID NO: 6 - protein, 234 aa, Artificial Sequence
  Light chain of anti-TROP2 antibody
MVLQTQVFISLLLWISGAYGDIQMTQSPSSLSASVGDRVTITCKASQDVSTAVAWYQQKPGKAPKLLIYSASYRYTGVPSRFSGSGSGTDFTLTISSLQPEDFAVYYCQQHYITPLTFGQGTKLEIKRTVAAPSVFIFPPSDEQLKSGTASVVCLLNNFYPREAKVQWKVDNALQSGNSQESVTEQDSKDSTYSLSSTLTLSKADYEKHKVYACEVTHQGLSSPVTKSFNRGEC

SEQ ID NO: 7 - protein, 471 aa, Artificial Sequence
  Heavy chain of anti-B7-H3 antibody
MKHLWFFLLLVAAPRWVLSQVQLVQSGAEVKKPGSSVKVSCKASGYTFTNYVMHWVRQAPGQGLEWMGYINPYNDDVKYNEKFKGRVTITADESTSTAYMELSSLRSEDTAVYYCARWGYYGSPLYYFDYWGQGTLVTVSSASTKGPSVFPLAPSSKSTSGGTAALGCLVKDYFPEPVTVSWNSGALTSGVHTFPAVLQSSGLYSLSSVVTVPSSSLGTQTYICNVNHKPSNTKVDKRVEPKSCDKTHTCPPCPAPELLGGPSVFLFPPKPKDTLMISRTPEVTCVVVDVSHEDPEVKFNWYVDGVEVHNAKTKPREEQYNSTYRVVSVLTVLHQDWLNGKEYKCKVSNKALPAPIEKTISKAKGQPREPQVYTLPPSREEMTKNQVSLTCLVKGFYPSDIAVEWESNGQPENNYKTTPPVLDSDGSFFLYSKLTVDKSRWQQGNVFSCSVMHEALHNHYTQKSLSLSPGK

SEQ ID NO: 8 - protein, 233 aa, Artificial Sequence
  Light chain of anti-B7-H3 antibody
MVLQTQVFISLLLWISGAYGEIVLTQSPATLSLSPGERATLSCRASSRLIYMHWYQQKPGQAPRPLIYATSNLASGIPARFSGSGSGTDFTLTISSLEPEDFAVYYCQQWNSNPPTFGQGTKVEIKRTVAAPSVFIFPPSDEQLKSGTASVVCLLNNFYPREAKVQWKVDNALQSGNSQESVTEQDSKDSTYSLSSTLTLSKADYEKHKVYACEVTHQGLSSPVTKSFNRGEC

SEQ ID NO: 9 - protein, 472 aa, Artificial Sequence
  Heavy chain of anti-GPR20 antibody
MKHLWFFLLLVAAPRWVLSEVQLVQSGAEVKKPGASVKVSCKASGYTFTSYYISWIRQAPGQGLKYMGFINPGSGHTNYNEKFKGRVTITADKSSSTATMELSSLRSEDTAVYYCARGAGGFLRIITKFDYWGQGTLVTVSSASTKGPSVFPLAPSSKSTSGGTAALGCLVKDYFPEPVTVSWNSGALTSGVHTFPAVLQSSGLYSLSSVVTVPSSSLGTQTYICNVNHKPSNTKVDKRVEPKSCDKTHTCPPCPAPELLGGPSVFLFPPKPKDTLMISRTPEVTCVVVDVSHEDPEVKFNWYVDGVEVHNAKTKPREEQYNSTYRVVSVLTVLHQDWLNGKEYKCKVSNKALPAPIEKTISKAKGQPREPQVYTLPPSREEMTKNQVSLTCLVKGFYPSDIAVEWESNGQPENNYKTTPPVLDSDGSFFLYSKLTVDKSRWQQGNVFSCSVMHEALHNHYTQKSLSLSPGK

SEQ ID NO: 10 - protein, 234 aa, Artificial Sequence
  Light chain of anti-GPR20 antibody
MVLQTQVFISLLLWISGAYGDTQLTQSPSSLSASVGDRVTITCRASKSVSTYIHWYQQKPGKQPKLLIYSAGNLESGVPSRFSGSGSGTDFTLTISSLQPEDFANYYCQQINELPYTFGQGTKVEIKRTVAAPSVFIFPPSDEQLKSGTASVVCLLNNFYPREAKVQWKVDNALQSGNSQESVTEQDSKDSTYSLSSTLTLSKADYEKHKVYACEVTHQGLSSPVTKSFNRGEC